European Patent Specification EP 3 783 102 B1, published September 13, 2023. Title: Amylase mutant having high specific activity and thermal stability, gene and application thereof. Applicant: Feed Research Institute, Chinese Academy of Agricultural Sciences. The sequence listing filed with the application follows.

SEQUENCE LISTING (6 sequences)

SEQ ID NO: 1 - protein, 485 aa, Bacillus amyloliquefaciens
AATNGTMMQYFEWYVPNDGQQWNRLRTDAPYLSSVGITAVWTPPAYKGTSQADVGYGPYDLYDLGEFNQKGTVRTKYGTKGELKSAVNTLHSNGIQVYGDVVMNHKAGADYTENVTAVEVNPSNRNQETSGEYNIQAWTGFNFPGRGTTYSNFKWQWFHFDGTDWDQSRSLSRIFKFRGTGKAWDWEVSSENGNYDYLMYADIDYDHPDVVNEMKKWGVWYANEVGLDGYRLDAVKHIKFSFLKDWVDNARAATGKEMFTVGEYWQNDLGALNNYLAKVNYNQSLFDAPLHYNFYAASTGGGYYDMRNILNNTLVASNPTKAVTLVENHDTQPGQSLESTVQPWFKPLAYAFILTRSGGYPSVFYGDMYGTKGTTTREIPALKSKIEPLLKARKDYAYGTQRDYIDNPDVIGWTREGDSTKAKSGLATVITDGPGGSKRMYVGTSNAGEIWYDLTGNRTDKITIGSDGYATFPVNGGSVSVWVQQ

SEQ ID NO: 2 - protein, 483 aa, Artificial Sequence
  synthesized mutant
AATNGTMMQYFEWYVPNDGQQWNRLRTDAPYLAEHGITAVWTPPAYKGTSQADVGYGPYDLYDLGEFNQKGTVRTKYGTKGELKSAVNTLHSNGIQVYGDVVMNHKAGADYTENVTAVEVNPSNRNQETSGEYNIQAWTGFNFPGRGTTYSNFKWQWFHFDGTDWDQSRSLSRIFKFTGKAWDWEVSSENGNYDYLMYADIDYDHPDVVNEMKKWGVWYANEVGLDGYRLDAVKHIKFSFLKDWVDNARAATGKEMFTVGEYWQNDLGALNNYLAKVNYNQSLFDAPLHYNFYAASTGGGYYDMRNILNNTLVASNPTKAVTLVENHDTQPGQSLESTVQPWFKPLAYAFILTRSGGYPSVFYGDMYGTKGTTTREIPALKSKIEPLLKARKDYAYGTQRDYIDNPDVIGWTREGDSTKAKSGLATVITDGPGGSKRMYVGTSNAGEIWYDLTGNRTDKITIGSDGYATFPVNGGSVSVWVQQ

SEQ ID NO: 3 - DNA, 50 bp, Artificial Sequence
  synthesized primer
ttacaaaaacatcagccgtaggatccgccgcaacgaacggaacaatgatg

SEQ ID NO: 4 - DNA, 54 bp, Artificial Sequence
  synthesized primer
gggacgtcgacttagtggtggtggtggtggtgctgctgaacccacactgagacg

SEQ ID NO: 5 - DNA, 51 bp, Artificial Sequence
  synthesized primer
gggttcagcagcaccaccaccaccaccactaagtcgacgtccccggggcag

SEQ ID NO: 6 - DNA, 50 bp, Artificial Sequence
  synthesized primer
attgttccgttcgttgcggcggatcctacggctgatgtttttgtaatcgg